European Patent Application EP 4 656 198 A2, published December 3, 2025. Title: USE OF GMI FROM GANODERMA LUCIDUM SPORES IN THE PREPARATION OF PHARMACEUTICALS AND FOOD PRODUCTS. Applicant: Titan Biological & Agricultural Technology Co., Limited. Application EP. The sequence listing filed with the application follows.

SEQUENCE LISTING (1 sequence)

SEQ ID NO: 1 - protein, 111 aa, unidentified
MSDTALIFTLAWNVKQLAFDYTPNWGRGRPSSFIDTVTFPTVLTDKAYTYRVVVSGKDLGVRPSYAVESDGSQKINFLEYNSGYGIADTNTIQVYVIDPDTGNNFIVAQWN